European Patent Application EP 4 393 946 A1, published July 3, 2024. Title: CDC PLATFORM ANTIBODY. Applicant: SUNSHINE GUOJIAN PHARMACEUTICAL (SHANGHAI) CO., LTD. The sequence listing filed with the application follows.

SEQUENCE LISTING (40 sequences)

SEQ ID NO: 1 - protein, 120 aa, synthetic construct
  source 1..120: note = heavy chain variable region of 50G12-Hu-IgG1
QVQLVQSGAEVKKPGASVKVSCKASGYTFNTYWMQWVRQAPGQGLEWMGAIYPGDGDITYNQKFKGRVTLTADKSTSTVYMELSSLRSEDTAVYYCAREGYYYGGALDYWGQGTLVTVSS

SEQ ID NO: 2 - protein, 108 aa, synthetic construct
  source 1..108: note = light chain variable region of 50G12-Hu-IgG1
DIQMTQSPSSLSASVGDRVTITCTASSSVSSSYLHWYQQKPGKAPKLWMYGTSNLASGVPSRFSGSGSGTDYTLTISSLQPEDFATYYCHRYHRSPWTFGQGTKVEIK

SEQ ID NO: 3 - protein, 330 aa, synthetic construct
  source 1..330: note = heavy chain constant region of Human IgG1
ASTKGPSVFPLAPSSKSTSGGTAALGCLVKDYFPEPVTVSWNSGALTSGVHTFPAVLQSSGLYSLSSVVTVPSSSLGTQTYICNVNHKPSNTKVDKKVEPKSCDKTHTCPPCPAPELLGGPSVFLFPPKPKDTLMISRTPEVTCVVVDVSHEDPEVKFNWYVDGVEVHNAKTKPREEQYNSTYRVVSVLTVLHQDWLNGKEYKCKVSNKALPAPIEKTISKAKGQPREPQVYTLPPSREEMTKNQVSLTCLVKGFYPSDIAVEWESNGQPENNYKTTPPVLDSDGSFFLYSKLTVDKSRWQQGNVFSCSVMHEALHNHYTQKSLSLSPGK

SEQ ID NO: 4 - protein, 107 aa, synthetic construct [sequence omitted]

SEQ ID NO: 5 - protein, 450 aa, synthetic construct
  source 1..450: note = heavy chain of 50G12-Hu-IgG1
QVQLVQSGAEVKKPGASVKVSCKASGYTFNTYWMQWVRQAPGQGLEWMGAIYPGDGDITYNQKFKGRVTLTADKSTSTVYMELSSLRSEDTAVYYCAREGYYYGGALDYWGQGTLVTVSSASTKGPSVFPLAPSSKSTSGGTAALGCLVKDYFPEPVTVSWNSGALTSGVHTFPAVLQSSGLYSLSSVVTVPSSSLGTQTYICNVNHKPSNTKVDKKVEPKSCDKTHTCPPCPAPELLGGPSVFLFPPKPKDTLMISRTPEVTCVVVDVSHEDPEVKFNWYVDGVEVHNAKTKPREEQYNSTYRVVSVLTVLHQDWLNGKEYKCKVSNKALPAPIEKTISKAKGQPREPQVYTLPPSREEMTKNQVSLTCLVKGFYPSDIAVEWESNGQPENNYKTTPPVLDSDGSFFLYSKLTVDKSRWQQGNVFSCSVMHEALHNHYTQKSLSLSPGK

SEQ ID NO: 6 - protein, 215 aa, synthetic construct
  source 1..215: note = light chain of 50G12-Hu-IgG1
DIQMTQSPSSLSASVGDRVTITCTASSSVSSSYLHWYQQKPGKAPKLWMYGTSNLASGVPSRFSGSGSGTDYTLTISSLQPEDFATYYCHRYHRSPWTFGQGTKVEIKRTVAAPSVFIFPPSDEQLKSGTASVVCLLNNFYPREAKVQWKVDNALQSGNSQESVTEQDSKDSTYSLSSTLTLSKADYEKHKVYACEVTHQGLSSPVTKSFNRGEC

SEQ ID NO: 7 - protein, 18 aa, synthetic construct
  source 1..18: note = IgM tail-piece
PTLYNVSLVMSDTAGTCY

SEQ ID NO: 8 - protein, 18 aa, synthetic construct
  source 1..18: note = Pep-CS
PTLYNVSLVMSDTAGTSY

SEQ ID NO: 9 - protein, 468 aa, synthetic construct
  source 1..468: note = heavy chain of 50G12-Hu-IgG1-Pep
QVQLVQSGAEVKKPGASVKVSCKASGYTFNTYWMQWVRQAPGQGLEWMGAIYPGDGDITYNQKFKGRVTLTADKSTSTVYMELSSLRSEDTAVYYCAREGYYYGGALDYWGQGTLVTVSSASTKGPSVFPLAPSSKSTSGGTAALGCLVKDYFPEPVTVSWNSGALTSGVHTFPAVLQSSGLYSLSSVVTVPSSSLGTQTYICNVNHKPSNTKVDKKVEPKSCDKTHTCPPCPAPELLGGPSVFLFPPKPKDTLMISRTPEVTCVVVDVSHEDPEVKFNWYVDGVEVHNAKTKPREEQYNSTYRVVSVLTVLHQDWLNGKEYKCKVSNKALPAPIEKTISKAKGQPREPQVYTLPPSREEMTKNQVSLTCLVKGFYPSDIAVEWESNGQPENNYKTTPPVLDSDGSFFLYSKLTVDKSRWQQGNVFSCSVMHEALHNHYTQKSLSLSPGKPTLYNVSLVMSDTAGTCY

SEQ ID NO: 10 - protein, 468 aa, synthetic construct
  source 1..468: note = heavy chain of 50G12-Hu-IgG1-Pep-CS
QVQLVQSGAEVKKPGASVKVSCKASGYTFNTYWMQWVRQAPGQGLEWMGAIYPGDGDITYNQKFKGRVTLTADKSTSTVYMELSSLRSEDTAVYYCAREGYYYGGALDYWGQGTLVTVSSASTKGPSVFPLAPSSKSTSGGTAALGCLVKDYFPEPVTVSWNSGALTSGVHTFPAVLQSSGLYSLSSVVTVPSSSLGTQTYICNVNHKPSNTKVDKKVEPKSCDKTHTCPPCPAPELLGGPSVFLFPPKPKDTLMISRTPEVTCVVVDVSHEDPEVKFNWYVDGVEVHNAKTKPREEQYNSTYRVVSVLTVLHQDWLNGKEYKCKVSNKALPAPIEKTISKAKGQPREPQVYTLPPSREEMTKNQVSLTCLVKGFYPSDIAVEWESNGQPENNYKTTPPVLDSDGSFFLYSKLTVDKSRWQQGNVFSCSVMHEALHNHYTQKSLSLSPGKPTLYNVSLVMSDTAGTSY

SEQ ID NO: 11 - protein, 5 aa, synthetic construct
  source 1..5: note = H-CDR1 of OKT10 heavy chain
RSWMN

SEQ ID NO: 12 - protein, 17 aa, synthetic construct
  source 1..17: note = H-CDR2 of OKT10 heavy chain
EINPDSSTINYTTSLKD

SEQ ID NO: 13 - protein, 7 aa, synthetic construct
  source 1..7: note = H-CDR3 of OKT10 heavy chain
YGNWFPY

SEQ ID NO: 14 - protein, 11 aa, synthetic construct
  source 1..11: note = L-CDR1 of OKT10 light chain
KASQNVDTNVA

SEQ ID NO: 15 - protein, 7 aa, synthetic construct
  source 1..7: note = L-CDR2 of OKT10 light chain
SASYRYS

SEQ ID NO: 16 - protein, 9 aa, synthetic construct
  source 1..9: note = L-CDR3 of OKT10 light chain
QQYDSYPLT

SEQ ID NO: 17 - protein, 11 aa, synthetic construct
  source 1..11: note = heavy chain framework region H-FR4 of OKT10
WGQGTLVTVSS

SEQ ID NO: 18 - protein, 10 aa, synthetic construct
  source 1..10: note = light chain framework region L-FR4 of OKT10
FGQGTKVEIK

SEQ ID NO: 19 - protein, 116 aa, synthetic construct
  source 1..116: note = heavy chain variable region of OKT10
EVKLQESGGGLVQPGGSLKLSCAASGFDFSRSWMNWVRQAPGKGLEWIGEINPDSSTINYTTSLKDKFIISRDNAKNTLYLQMTKVRSEDTALYYCARYGNWFPYWGQGTLVTVSA

SEQ ID NO: 20 - protein, 107 aa, synthetic construct
  source 1..107: note = light chain variable region of OKT10
DIVMTQSPKIMPTSVGDRVSVTCKASQNVDTNVAWYQQKPGQSPKALIYSASYRYSGVPDRFTGSGSGTDFTLTITNVQSEDLAEYFCQQYDSYPLTFGAGTKLDLK

SEQ ID NO: 21 - protein, 116 aa, synthetic construct
  source 1..116: note = Humanized Heavy Chain Variable Region of OKT10
EVQLVESGGGLVQPGGSLRLSCAASGFDFSRSWMNWVRQAPGKGLEWVSEINPDSSTINYTTSLKDRFTISRDNAKNSLYLQMNSLRAEDTAVYYCARYGNWFPYWGQGTLVTVSS

SEQ ID NO: 22 - protein, 107 aa, synthetic construct
  source 1..107: note = Humanized Light Chain Variable Region of OKT10
DIQMTQSPSSLSASVGDRVTITCKASQNVDTNVAWYQQKPGKAPKALIYSASYRYSGVPSRFSGSGSGTDFTLTISSLQPEDFATYYCQQYDSYPLTFGQGTKVEIK

SEQ ID NO: 23 - protein, 446 aa, synthetic construct
  source 1..446: note = humanized heavy chain of OKT10
EVQLVESGGGLVQPGGSLRLSCAASGFDFSRSWMNWVRQAPGKGLEWVSEINPDSSTINYTTSLKDRFTISRDNAKNSLYLQMNSLRAEDTAVYYCARYGNWFPYWGQGTLVTVSSASTKGPSVFPLAPSSKSTSGGTAALGCLVKDYFPEPVTVSWNSGALTSGVHTFPAVLQSSGLYSLSSVVTVPSSSLGTQTYICNVNHKPSNTKVDKKVEPKSCDKTHTCPPCPAPELLGGPSVFLFPPKPKDTLMISRTPEVTCVVVDVSHEDPEVKFNWYVDGVEVHNAKTKPREEQYNSTYRVVSVLTVLHQDWLNGKEYKCKVSNKALPAPIEKTISKAKGQPREPQVYTLPPSREEMTKNQVSLTCLVKGFYPSDIAVEWESNGQPENNYKTTPPVLDSDGSFFLYSKLTVDKSRWQQGNVFSCSVMHEALHNHYTQKSLSLSPGK

SEQ ID NO: 24 - protein, 214 aa, synthetic construct
  source 1..214: note = humanized light chain of OKT10
DIQMTQSPSSLSASVGDRVTITCKASQNVDTNVAWYQQKPGKAPKALIYSASYRYSGVPSRFSGSGSGTDFTLTISSLQPEDFATYYCQQYDSYPLTFGQGTKVEIKRTVAAPSVFIFPPSDEQLKSGTASVVCLLNNFYPREAKVQWKVDNALQSGNSQESVTEQDSKDSTYSLSSTLTLSKADYEKHKVYACEVTHQGLSSPVTKSFNRGEC

SEQ ID NO: 25 - protein, 464 aa, synthetic construct
  source 1..464: note = heavy chain of OKT10-Hu-IgG1-Pep-CS
EVQLVESGGGLVQPGGSLRLSCAASGFDFSRSWMNWVRQAPGKGLEWVSEINPDSSTINYTTSLKDRFTISRDNAKNSLYLQMNSLRAEDTAVYYCARYGNWFPYWGQGTLVTVSSASTKGPSVFPLAPSSKSTSGGTAALGCLVKDYFPEPVTVSWNSGALTSGVHTFPAVLQSSGLYSLSSVVTVPSSSLGTQTYICNVNHKPSNTKVDKKVEPKSCDKTHTCPPCPAPELLGGPSVFLFPPKPKDTLMISRTPEVTCVVVDVSHEDPEVKFNWYVDGVEVHNAKTKPREEQYNSTYRVVSVLTVLHQDWLNGKEYKCKVSNKALPAPIEKTISKAKGQPREPQVYTLPPSREEMTKNQVSLTCLVKGFYPSDIAVEWESNGQPENNYKTTPPVLDSDGSFFLYSKLTVDKSRWQQGNVFSCSVMHEALHNHYTQKSLSLSPGKPTLYNVSLVMSDTAGTSY

SEQ ID NO: 26 - protein, 122 aa, synthetic construct [sequence omitted]

SEQ ID NO: 27 - protein, 107 aa, synthetic construct [sequence omitted]

SEQ ID NO: 28 - protein, 120 aa, synthetic construct [sequence omitted]

SEQ ID NO: 29 - protein, 107 aa, synthetic construct [sequence omitted]

SEQ ID NO: 30 - protein, 258 aa, Macaca fascicularis
  source 1..258: note = Cynomolgus monkey CD38 extracellular
LPRWRQQWSGSGTTSRFPETVLARCVKYTEVHPEMRHVDCQSVWDAFKGAFISKYPCNITEEDYQPLVKLGTQTVPCNKTLLWSRIKDLAHQFTQVQRDMFTLEDMLLGYLADDLTWCGEFNTFEINYQSCPDWRKDCSNNPVSVFWKTVSRRFAETACGVVHVMLNGSRSKIFDKNSTFGSVEVHNLQPEKVQALEAWVIHGGREDSRDLCQDPTIKELESIISKRNIRFFCKNIYRPDKFLQCVKNPEDSSCLSGI

SEQ ID NO: 31 - protein, 348 aa, synthetic construct
  source 1..348: note = Human IgG1-Pep-CS
ASTKGPSVFPLAPSSKSTSGGTAALGCLVKDYFPEPVTVSWNSGALTSGVHTFPAVLQSSGLYSLSSVVTVPSSSLGTQTYICNVNHKPSNTKVDKKVEPKSCDKTHTCPPCPAPELLGGPSVFLFPPKPKDTLMISRTPEVTCVVVDVSHEDPEVKFNWYVDGVEVHNAKTKPREEQYNSTYRVVSVLTVLHQDWLNGKEYKCKVSNKALPAPIEKTISKAKGQPREPQVYTLPPSREEMTKNQVSLTCLVKGFYPSDIAVEWESNGQPENNYKTTPPVLDSDGSFFLYSKLTVDKSRWQQGNVFSCSVMHEALHNHYTQKSLSLSPGKPTLYNVSLVMSDTAGTSY

SEQ ID NO: 32 - protein, 330 aa, synthetic construct
  SITE 192: note = Xaa is E, F , H, C, D, N , Q ,R, S , T, K, W or Y
  source 1..330: note = IgG1-L309X
ASTKGPSVFPLAPSSKSTSGGTAALGCLVKDYFPEPVTVSWNSGALTSGVHTFPAVLQSSGLYSLSSVVTVPSSSLGTQTYICNVNHKPSNTKVDKKVEPKSCDKTHTCPPCPAPELLGGPSVFLFPPKPKDTLMISRTPEVTCVVVDVSHEDPEVKFNWYVDGVEVHNAKTKPREEQYNSTYRVVSVLTVXHQDWLNGKEYKCKVSNKALPAPIEKTISKAKGQPREPQVYTLPPSREEMTKNQVSLTCLVKGFYPSDIAVEWESNGQPENNYKTTPPVLDSDGSFFLYSKLTVDKSRWQQGNVFSCSVMHEALHNHYTQKSLSLSPGK

SEQ ID NO: 33 - protein, 450 aa, synthetic construct
  source 1..450: note = 50G12-Hu-IgG1-L309W-E345R
QVQLVQSGAEVKKPGASVKVSCKASGYTFNTYWMQWVRQAPGQGLEWMGAIYPGDGDITYNQKFKGRVTLTADKSTSTVYMELSSLRSEDTAVYYCAREGYYYGGALDYWGQGTLVTVSSASTKGPSVFPLAPSSKSTSGGTAALGCLVKDYFPEPVTVSWNSGALTSGVHTFPAVLQSSGLYSLSSVVTVPSSSLGTQTYICNVNHKPSNTKVDKKVEPKSCDKTHTCPPCPAPELLGGPSVFLFPPKPKDTLMISRTPEVTCVVVDVSHEDPEVKFNWYVDGVEVHNAKTKPREEQYNSTYRVVSVLTVWHQDWLNGKEYKCKVSNKALPAPIEKTISKAKGQPRRPQVYTLPPSREEMTKNQVSLTCLVKGFYPSDIAVEWESNGQPENNYKTTPPVLDSDGSFFLYSKLTVDKSRWQQGNVFSCSVMHEALHNHYTQKSLSLSPGK

SEQ ID NO: 34 - protein, 330 aa, synthetic construct
  source 1..330: note = IgG1-L309W-E345R
ASTKGPSVFPLAPSSKSTSGGTAALGCLVKDYFPEPVTVSWNSGALTSGVHTFPAVLQSSGLYSLSSVVTVPSSSLGTQTYICNVNHKPSNTKVDKKVEPKSCDKTHTCPPCPAPELLGGPSVFLFPPKPKDTLMISRTPEVTCVVVDVSHEDPEVKFNWYVDGVEVHNAKTKPREEQYNSTYRVVSVLTVWHQDWLNGKEYKCKVSNKALPAPIEKTISKAKGQPRRPQVYTLPPSREEMTKNQVSLTCLVKGFYPSDIAVEWESNGQPENNYKTTPPVLDSDGSFFLYSKLTVDKSRWQQGNVFSCSVMHEALHNHYTQKSLSLSPGK

SEQ ID NO: 35 - protein, 5 aa, synthetic construct
  source 1..5: note = H-CDR1 of 50G12 heavy chain
TYWMQ

SEQ ID NO: 36 - protein, 17 aa, synthetic construct
  source 1..17: note = H-CDR2 of 50G12 heavy chain
AIYPGDGDITYNQKFKG

SEQ ID NO: 37 - protein, 11 aa, synthetic construct
  source 1..11: note = H-CDR3 of 50G12 heavy chain
EGYYYGGALDY

SEQ ID NO: 38 - protein, 12 aa, synthetic construct
  source 1..12: note = L-CDR1 of 50G12 light chain
TASSSVSSSYLH

SEQ ID NO: 39 - protein, 7 aa, synthetic construct
  source 1..7: note = L-CDR2 of 50G12 light chain
GTSNLAS

SEQ ID NO: 40 - protein, 9 aa, synthetic construct
  source 1..9: note = L-CDR3 of 50G12 light chain
HRYHRSPWT